European Patent Specification EP 3 515 928 B1, published January 28, 2026. Title: UNSTRUCTURED NON-REPETITIVE POLYPEPTIDES HAVING LCST BEHAVIOR. Applicant: DUKE UNIVERSITY. The sequence listing filed with the application follows.

SEQUENCE LISTING (23 sequences)

SEQ ID NO: 1 - protein, 10 aa, Homo sapien
GAGVPGVGVP

SEQ ID NO: 2 - protein, 25 aa, Homo sapien
GVGVPGVGVPGAGVPGVGVPGVGVP

SEQ ID NO: 3 - protein, 200 aa, Homo sapien
GVGVPGVGVPGAGVPGVGVPGVGVPGVGVPGVGVPGAGVPGVGVPGVGVPGVGVPGVGVPGAGVPGVGVPGVGVPGVGVPGVGVPGAGVPGVGVPGVGVPGVGVPGVGVPGAGVPGVGVPGVGVPGVGVPGVGVPGAGVPGVGVPGVGVPGVGVPGVGVPGAGVPGVGVPGVGVPGVGVPGVGVPGAGVPGVGVPGVGVP

SEQ ID NO: 4 - protein, 200 aa, Homo sapien
GAGVPGVGVPGAGVPGVGVPGAGVPGVGVPGAGVPGVGVPGAGVPGVGVPGAGVPGVGVPGAGVPGVGVPGAGVPGVGVPGAGVPGVGVPGAGVPGVGVPGAGVPGVGVPGAGVPGVGVPGAGVPGVGVPGAGVPGVGVPGAGVPGVGVPGAGVPGVGVPGAGVPGVGVPGAGVPGVGVPGAGVPGVGVPGAGVPGVGVP

SEQ ID NO: 5 - protein, 400 aa, Homo sapien
GVGVPGVGVPGAGVPGVGVPGVGVPGVGVPGVGVPGAGVPGVGVPGVGVPGVGVPGVGVPGAGVPGVGVPGVGVPGVGVPGVGVPGAGVPGVGVPGVGVPGVGVPGVGVPGAGVPGVGVPGVGVPGVGVPGVGVPGAGVPGVGVPGVGVPGVGVPGVGVPGAGVPGVGVPGVGVPGVGVPGVGVPGAGVPGVGVPGVGVPGVGVPGVGVPGAGVPGVGVPGVGVPGVGVPGVGVPGAGVPGVGVPGVGVPGVGVPGVGVPGAGVPGVGVPGVGVPGVGVPGVGVPGAGVPGVGVPGVGVPGVGVPGVGVPGAGVPGVGVPGVGVPGVGVPGVGVPGAGVPGVGVPGVGVPGVGVPGVGVPGAGVPGVGVPGVGVPGVGVPGVGVPGAGVPGVGVPGVGVP

SEQ ID NO: 6 - protein, 400 aa, Homo sapien
GAGVPGVGVPGAGVPGVGVPGAGVPGVGVPGAGVPGVGVPGAGVPGVGVPGAGVPGVGVPGAGVPGVGVPGAGVPGVGVPGAGVPGVGVPGAGVPGVGVPGAGVPGVGVPGAGVPGVGVPGAGVPGVGVPGAGVPGVGVPGAGVPGVGVPGAGVPGVGVPGAGVPGVGVPGAGVPGVGVPGAGVPGVGVPGAGVPGVGVPGAGVPGVGVPGAGVPGVGVPGAGVPGVGVPGAGVPGVGVPGAGVPGVGVPGAGVPGVGVPGAGVPGVGVPGAGVPGVGVPGAGVPGVGVPGAGVPGVGVPGAGVPGVGVPGAGVPGVGVPGAGVPGVGVPGAGVPGVGVPGAGVPGVGVPGAGVPGVGVPGAGVPGVGVPGAGVPGVGVPGAGVPGVGVPGAGVPGVGVP

SEQ ID NO: 7 - protein, 200 aa, Artificial sequence
  Synthetic
PGGGVPGGVPGAVPGVPGAVVPVVGGVPGVVGVPGGVVPVGVVVPGVPVGVPGVPVVGGGVPAGGVVPGGGVPVGGGVVPGVGVVPGGVPVVVGGGVGVPGVVPGVPGVGVPVGGVPGGGVVVPGGVGVPVVGVVPGAPGVPGVPGGVGGVPVGVGVPGGGAPGVVPGGAVPGGAPVGGVGGGVPGVGGVPGAPGGVPGG

SEQ ID NO: 8 - protein, 200 aa, Artificial sequence
  Synthetic
PGGVPGVPAGGGAGVPGVPGAPAGGGAPGVAPGGVVPGVPGVAPVVGGGAPGGVPGAVPGVPGGVPGGVVVPGGGVGAPGGVAPVGGGVPVVGGVPVGGVAPGVPVGVPGVGVGVGVPVGGGVGGVPGVVPAGVPGGGVAGVVPVGGVPVVVGAPGGGVGVPGAPGAGGVPGGAPGAPGVVAPGGVPVGVVVPGVVPGGG

SEQ ID NO: 9 - protein, 400 aa, Artificial sequence
  Synthetic
PGGVPGVGGGVPGVPGAPGVVPGVVVPGGVVPVGGVPGVPVVGGGVPVGGGVGGVPGAPGGGVPGAPVGGVPVGGVVPGVGVPGAGGGVPGGVGVVPVGGGAPGGVPGVVPGVPVGGVPAGVVPGGVGVGGGVVPGVVGVPGGGVGGGVGVPGGAPGGGVVGGGVPGGGVVPVVGGVPGAVPGVPGVVVPVGGGVVPVGVPGGVVVPGVPGGVVGVPVVGVPGVGVVPGVPGVPVGVGVVVPGVVPVGVGVPGVPGGGVPGVGVPVGGAPGVPGVPGVAVPGVVPGGAPGVPVGVVPVGVVPGGGVGVVPGGVPGGVPGVPAGVPVGVPVGGVGGVVPGGGAPGVGVGVPAGVPGGVPVGVGGVPGGVVPGVPAGGGVPVGVPGVGGVPVGAPGVPGGVP

SEQ ID NO: 10 - protein, 400 aa, Artificial sequence
  Synthetic
PAGAVPGGVPVAGGVPVGAGVVAPGAPVGGAPGVVGVPGGGVPGVPVVGVGVGVPVGGGVGVVPAGGGAPGGVGVVVPGVVPGAPAGGVPGVAPGGVGGVPGVVPGGGVVPGVAPGVPGVPGGVPVGVPVGAAPGGGVPAVGVPGVGGGVPVVGAGAPGGVPGVAVPGAPGGVPVGGVPGGGVGGVVPGGVPGAPVGVVPGVGVVPGVPAGVGVPGAPGAPGGGVPGGGAPVGGAGGVPGGVPGVPGAPGVGVPGVGVPVGVPGVPGVPVGGGAGVPGGVAPGVAVPGGVGVPVVGGVPGAVPGVPGVGGAPGVPGGGVVGVGVPGGVVPGVPGAGAPGGGAPGAPVGVPGGAPGVVPGVGGVPGAGGGVVGGGVVPVGGGVVPGAPGGAPVGGVVGGVP

SEQ ID NO: 11 - protein, 240 aa, Artificial sequence
  Synthetic
PVGVPGVGGAPVVVGGAPVGVGGAGGVVPGAPVGAVAGVGAPGGAVPAGGAPGVGAPGVVPGAVPGVGVGGVGGGVVVPVVVGVGGVPAGAVPVGGVAPVGVPVGAGGGAPAGGVPVAVGVPVVGGGVPGVGVVGVAPGAPGAGVGVVAGAGAAAVAPVGVAPGVPGVPGAVVGVPGGVAPAVVVGAVPGVVGVVPVGAPVVAGGVAVAPVGGAVPGVPGGVPGGGAPGAPVVGVPVGVP

SEQ ID NO: 12 - protein, 240 aa, Artificial sequence
  Synthetic
PVGSPGSVPGVVPVSGVVVGGGSVPGSSPVVGVPSGVPVGSPVVGGGVSPGVGVPGVVVPGVPVGGGVGVPGGGVVGGVPVVVGVSVPSGVSPGGGVVVPVGSVSSGVPVVSVVGVSVVPGSVPVGSPSSGVPGVVPGSPGGVVGSSVPSGSGGVSVPVGVGGSGVPGVPGSGSVVPVGVSPVGGGSGSGVGSGSPGGSVPGGSPGVVPVGSPGVGGVPGVVGGSGSPGVPGGVGVGVPG

SEQ ID NO: 13 - protein, 240 aa, Artificial sequence
  Synthetic
PVGTPGTVPGGVVPVGVTPVGGGTGTPTTVTVVGGVVVPGVPGGGTPGVPVGTPVVGGVGVGTGTPGGTVPGGTPGVVPGTPGGVVPGTTVPTGTGTTPVVGVPTVGGVTPGVGGVPVVVGTGVPGVPVGGGVGVVGVVVPGTVPVGVPGVVGGTVPVGTPTTGVPGVVPTGVTPGGVGVPGGGVVGGVVPGVTVPVGTVTTGVPVVTVGVVVPVGTVGGVVVGGGTTPGGVPGTPGVGG

SEQ ID NO: 14 - protein, 240 aa, Artificial sequence
  Synthetic
GAVVVPGGAVGVPAGAVGGVGGVLVPAVGAVPGGGVPAVGVPVAGVVPGGLPGGAGVGALGAAAPGGVPVGAALPGVAGVAPGGGLPGLGAGAGLGLAGALVLPGLGGVPGVPGGGLLPGGVPLLGLPGVPAGLPGVLPVGLLLPGAPGVPALGVPLGVPGVAPGLPGAGGLPGVGAPGLLPVGGAPAALGGLGLPGGGALGLLAPGGALVPGVGGVAPVAAGALLPGGAPLGVPALLAL

SEQ ID NO: 15 - protein, 240 aa, Artificial sequence
  Synthetic
SSGSSGSGFFSGGVPSGGGVVFVPSFFGFFPSGSGGVVPGVPGGGVGVPGFVGVPVGGFPVGVPGVFVPSVVGVPGFFVFPGVPGGSSSPGSPFGVFGGGSSGGGFPFGSSPGVVVSPGFGFGVPFGVPVGGSVFFFPFGGGFPGGFPSGSFGVPGGGFVVPFGVSPGSPGFVPSFGSPGGFGGFSPFSSGVGSPGGVPGVGVVSPGFPGGSPFGFPGSPGGSFGGSPSVFGSGSPGSFP

SEQ ID NO: 16 - protein, 240 aa, Artificial sequence
  Synthetic
AAGGTGFFTGGAPGGTPTAFGGFTPFTFAGGGAPGFFAFPGAPGTFPTFGAPGAAPFGTTPGTFFGFPGGTPGTPGAATPGFFGAFGFPGAFATFGFPGGGAGAAPAGTPGAPTAAGATTPGAGGTTGGAPTGGGFAPTFFGFFPTGTGGAAPGAPGGGTTTFPGATPFGFPGTGTPGTFGAPGGGFFPGAGFGGGAPGAPAAAGGGTPGTATPGTFPTGAGTFPGTFPFGGGFPGGFPT

SEQ ID NO: 17 - protein, 240 aa, Artificial sequence
  Synthetic
TILPGIGLPGGLPLTIGGILPILLGTTIGGIPGGGIIPGIGGGIPILTLLILPTGLPGTPLTTGTPGITGLGTPLGIGLIGTGIPGGGTGIPTGIPGTTLPGIPTLGGGIPLIGTPGGIGTIGIPGTGTIIGIPGGGLLLIPGITPLIGLPGGTPGTPGGGTGTTPTGLPGILLPGGLPGIPTGTPGTGTPIGGLLILLTLPGLPGLGLPGLIPLGTGLTGGTPTGGIPGGIGIPGILTT

SEQ ID NO: 18 - protein, 240 aa, Artificial sequence
  Synthetic
PGTYPGYGYVYPTTGGIPGGVVPGGGTKLVPGKGKGGAKAPGTVPVGAGGGKIVPIYGIAPGKYGYPGGGIVPGITTPGLPTGKKPYGGVPVLYGKLPGAPGIPTAGAPGYIAPGVPGGLVKGGTGIAPLGVILVYIGVGGIKGGALPTGGLYPGAGTPGYPVGGGAPAGGIALKPGITPGTAAPGLPGKGGKYTYPGGAPGGTGGVPGYPGLALKLGIPTKGGGIGLPYIGLLPGKPGG

SEQ ID NO: 19 - protein, 6 aa, Artificial sequence
  Synthetic
MSKGPG

SEQ ID NO: 20 - protein, 3 aa, Artificial sequence
  Synthetic
GWP

SEQ ID NO: 21 - protein, 15 aa, Artificial sequence
  Synthetic
GGGGSGGGGSGGGGS

SEQ ID NO: 22 - protein, 19 aa, Artificial sequence
  Synthetic
PQPQPKPQPKPEPEPQPQG

SEQ ID NO: 23 - protein, 5 aa, Artificial sequence
  Synthetic
  Xaa (4)..(4): any amino acid except proline
VPGXG